European Patent Specification EP 3 430 129 B1, published October 25, 2023. Title: Colony Forming Medium and Use Thereof. Applicant: Cynata Therapeutics Limited. The sequence listing filed with the application follows.

SEQUENCE LISTING (8 sequences)

SEQ ID NO: 1 - protein, 116 aa, Homo sapiens [sequence omitted]

SEQ ID NO: 2 - protein, 106 aa, Homo sapiens
KKNKNCRRHSLYVDFSDVGWNDWIVAPPGYQAFYCHGDCPFPLADHLNSTNHAIVQTLVNSVNSSIPKACCVPTELSAISMLYLDEYDKVVLKNYQEMVVEGCGCR

SEQ ID NO: 3 - protein, 1057 aa, Homo sapiens
QLSYGYDEKSTGGISVPGPMGPSGPRGLPGPPGAPGPQGFQGPPGEPGEPGASGPMGPRGPPGPPGKNGDDGEAGKPGRPGERGPPGPQGARGLPGTAGLPGMKGHRGFSGLDGAKGDAGPAGPKGEPGSPGENGAPGQMGPRGLPGERGRPGAPGPAGARGNDGATGAAGPPGPTGPAGPPGFPGAVGAKGEAGPQGPRGSEGPQGVRGEPGPPGPAGAAGPAGNPGADGQPGAKGANGAPGIAGAPGFPGARGPSGPQGPGGPPGPKGNSGEPGAPGSKGDTGAKGEPGPVGVQGPPGPAGEEGKRGARGEPGPTGLPGPPGERGGPGSRGFPGADGVAGPKGPAGERGSPGPAGPKGSPGEAGRPGEAGLPGAKGLTGSPGSPGPDGKTGPPGPAGQDGRPGPPGPPGARGQAGVMGFPGPKGAAGEPGKAGERGVPGPPGAVGPAGKDGEAGAQGPPGPAGPAGERGEQGPAGSPGFQGLPGPAGPPGEAGKPGEQGVPGDLGAPGPSGARGERGFPGERGVQGPPGPAGPRGANGAPGNDGAKGDAGAPGAPGSQGAPGLQGMPGERGAAGLPGPKGDRGDAGPKGADGSPGKDGVRGLTGPIGPPGPAGAPGDKGESGPSGPAGPTGARGAPGDRGEPGPPGPAGFAGPPGADGQPGAKGEPGDAGAKGDAGPPGPAGPAGPPGPIGNVGAPGAKGARGSAGPPGATGFPGAAGRVGPPGPSGNAGPPGPPGPAGKEGGKGPRGETGPAGRPGEVGPPGPPGPAGEKGSPGADGPAGAPGTPGPQGIAGQRGVVGLPGQRGERGFPGLPGPSGEPGKQGPSGASGERGPPGPMGPPGLAGPPGESGREGAPGAEGSPGRDGSPGAKGDRGETGPAGPPGAPGAPGAPGPVGPAGKSGDRGETGPAGPAGPVGPVGARGPAGPQGPRGDKGETGEQGDRGIKGHRGFSGLQGPPGPPGSPGEQGPSGASGPAGPRGPPGSAGAPGKDGLNGLPGPIGPPGPRGRTGDAGPVGPPGPPGPPGPPGPPSAGFDFSFLPQPPQEKAHDGGRYYRA

SEQ ID NO: 4 - protein, 1497 aa, Homo sapiens
GERGFPGIPGTPGPPGLPGLQGPVGPPGFTGPPGPPGPPGPPGEKGQMGLSFQGPKGDKGDQGVSGPPGVPGQAQVQEKGDFATKGEKGQKGEPGFQGMPGVGEKGEPGKPGPRGKPGKDGDKGEKGSPGFPGEPGYPGLIGRQGPQGEKGEAGPPGPPGIVIGTGPLGEKGERGYPGTPGPRGEPGPKGFPGLPGQPGPPGLPVPGQAGAPGFPGERGEKGDRGFPGTSLPGPSGRDGLPGPPGSPGPPGQPGYTNGIVECQPGPPGDQGPPGIPGQPGFIGEIGEKGQKGESCLICDIDGYRGPPGPQGPPGEIGFPGQPGAKGDRGLPGRDGVAGVPGPQGTPGLIGQPGAKGEPGEFYFDLRLKGDKGDPGFPGQPGMPGRAGSPGRDGHPGLPGPKGSPGSVGLKGERGPPGGVGFPGSRGDTGPPGPPGYGPAGPIGDKGQAGFPGGPGSPGLPGPKGEPGKIVPLPGPPGAEGLPGSPGFPGPQGDRGFPGTPGRPGLPGEKGAVGQPGIGFPGPPGPKGVDGLPGDMGPPGTPGRPGFNGLPGNPGVQGQKGEPGVGLPGLKGLPGLPGIPGTPGEKGSIGVPGVPGEHGAIGPPGLQGIRGEPGPPGLPGSVGSPGVPGIGPPGARGPPGGQGPPGLSGPPGIKGEKGFPGFPGLDMPGPKGDKGAQGLPGITGQSGLPGLPGQQGAPGIPGFPGSKGEMGVMGTPGQPGSPGPVGAPGLPGEKGDHGFPGSSGPRGDPGLKGDKGDVGLPGKPGSMDKVDMGSMKGQKGDQGEKGQIGPIGEKGSRGDPGTPGVPGKDGQAGQPGQPGPKGDPGISGTPGAPGLPGPKGSVGGMGLPGTPGEKGVPGIPGPQGSPGLPGDKGAKGEKGQAGPPGIGIPGLRGEKGDQGIAGFPGSPGEKGEKGSIGIPGMPGSPGLKGSPGSVGYPGSPGLPGEKGDKGLPGLDGIPGVKGEAGLPGTPGPTGPAGQKGEPGSDGIPGSAGEKGEPGLPGRGFPGFPGAKGDKGSKGEVGFPGLAGSPGIPGSKGEQGFMGPPGPQGQPGLPGSPGHATEGPKGDRGPQGQPGLPGLPGPMGPPGLPGIDGVKGDKGNPGWPGAPGVPGPKGDPGFQGMPGIGGSPGITGSKGDMGPPGVPGFQGPKGLPGLQGIKGDQGDQGVPGAKGLPGPPGPPGPYDIIKGEPGLPGPEGPPGLKGLQGLPGPKGQQGVTGLVGIPGPPGIPGFDGAPGQKGEMGPAGPTGPRGFPGPPGPDGLPGSMGPPGTPSVDHGFLVTRHSQTIDDPQCPSGTKILYHGYSLLYVQGNERAHGQDLGTAGSCLRKFSTMPFLFCNINNVCNFASRNDYSYWLSTPEPMPMSMAPITGENIRPFISRCAVCEAPAMVMAVHSQTIQIPPCPSGWSSLWIGYSFVMHTSAGAEGSGQALASPGSCLEEFRSAPFIECHGRGTCNYYANAYSFWLATIERSEMFKKPTPSTLKAGELRTHVSRCQVCMRRT

SEQ ID NO: 5 - protein, 288 aa, Homo sapiens
MVGVGGGDVEDVTPRPGGCQISGRGARGCNGIPGAAAWEAALPRRRPRRHPSVNPRSRAAGSPRTRGRRTEERPSGSRLGDRGRGRALPGGRLGGRGRGRAPERVGGRGRGRGTAAPRAAPAARGSRPGPAGTMAAGSITTLPALPEDGGSGAFPPGHFKDPKRLYCKNGGFFLRIHPDGRVDGVREKSDPHIKLQLQAEERGVVSIKGVCANRYLAMKEDGRLLASKCVTDECFFFERLESNNYNTYRSRKYTSWYVALKRTGQYKLGSKTGPGQKAILFLPMSAKS

SEQ ID NO: 6 - protein, 2415 aa, Homo sapiens
QAQQMVQPQSPVAVSQSKPGCYDNGKHYQINQQWERTYLGNALVCTCYGGSRGFNCESKPEAEETCFDKYTGNTYRVGDTYERPKDSMIWDCTCIGAGRGRISCTIANRCHEGGQSYKIGDTWRRPHETGGYMLECVCLGNGKGEWTCKPIAEKCFDHAAGTSYVVGETWEKPYQGWMMVDCTCLGEGSGRITCTSRNRCNDQDTRTSYRIGDTWSKKDNRGNLLQCICTGNGRGEWKCERHTSVQTTSSGSGPFTDVRAAVYQPQPHPQPPPYGHCVTDSGVVYSVGMQWLKTQGNKQMLCTCLGNGVSCQETAVTQTYGGNSNGEPCVLPFTYNGRTFYSCTTEGRQDGHLWCSTTSNYEQDQKYSFCTDHTVLVQTRGGNSNGALCHFPFLYNNHNYTDCTSEGRRDNMKWCGTTQNYDADQKFGFCPMAAHEEICTTNEGVMYRIGDQWDKQHDMGHMMRCTCVGNGRGEWTCIAYSQLRDQCIVDDITYNVNDTFHKRHEEGHMLNCTCFGQGRGRWKCDPVDQCQDSETGTFYQIGDSWEKYVHGVRYQCYCYGRGIGEWHCQPLQTYPSSSGPVEVFITETPSQPNSHPIQWNAPQPSHISKYILRWRPKNSVGRWKEATIPGHLNSYTIKGLKPGVVYEGQLISIQQYGHQEVTRFDFTTTSTSTPVTSNTVTGETTPFSPLVATSESVTEITASSFVVSWVSASDTVSGFRVEYELSEEGDEPQYLDLPSTATSVNIPDLLPGRKYIVNVYQISEDGEQSLILSTSQTTAPDAPPDPTVDQVDDTSIVVRWSRPQAPITGYRIVYSPSVEGSSTELNLPETANSVTLSDLQPGVQYNITIYAVEENQESTPVVIQQETTGTPRSDTVPSPRDLQFVEVTDVKVTIMWTPPESAVTGYRVDVIPVNLPGEHGQRLPISRNTFAEVTGLSPGVTYYFKVFAVSHGRESKPLTAQQTTKLDAPTNLQFVNETDSTVLVRWTPPRAQITGYRLTVGLTRRGQPRQYNVGPSVSKYPLRNLQPASEYTVSLVAIKGNQESPKATGVFTTLQPGSSIPPYNTEVTETTIVITWTPAPRIGFKLGVRPSQGGEAPREVTSDSGSIVVSGLTPGVEYVYTIQVLRDGQERDAPIVNKVVTPLSPPTNLHLEANPDTGVLTVSWERSTTPDITGYRITTTPTNGQQGNSLEEVVHADQSSCTFDNLSPGLEYNVSVYTVKDDKESVPISDTIIPEVPQLTDLSFVDITDSSIGLRWTPLNSSTIIGYRITVVAAGEGIPIFEDFVDSSVGYYTVTGLEPGIDYDISVITLINGGESAPTTLTQQTAVPPPTDLRFTNIGPDTMRVTWAPPPSIDLTNFLVRYSPVKNEEDVAELSISPSDNAVVLTNLLPGTEYVVSVSSVYEQHESTPLRGRQKTGLDSPTGIDFSDITANSFTVHWIAPRATITGYRIRHHPEHFSGRPREDRVPHSRNSITLTNLTPGTEYVVSIVALNGREESPLLIGQQSTVSDVPRDLEVVAATPTSLLISWDAPAVTVRYYRITYGETGGNSPVQEFTVPGSKSTATISGLKPGVDYTITVYAVTGRGDSPASSKPISINYRTEIDKPSQMQVTDVQDNSISVKWLPSSSPVTGYRVTTTPKNGPGPTKTKTAGPDQTEMTIEGLQPTVEYVVSVYAQNPSGESQPLVQTAVTNIDRPKGLAFTDVDVDSIKIAWESPQGQVSRYRVTYSSPEDGIHELFPAPDGEEDTAELQGLRPGSEYTVSVVALHDDMESQPLIGTQSTAIPAPTDLKFTQVTPTSLSAQWTPPNVQLTGYRVRVTPKEKTGPMKEINLAPDSSSVVVSGLMVATKYEVSVYALKDTLTSRPAQGVVTTLENVSPPRRARVTDATETTITISWRTKTETITGFQVDAVPANGQTPIQRTIKPDVRSYTITGLQPGTDYKIYLYTLNDNARSSPVVIDASTAIDAPSNLRFLATTPNSLLVSWQPPRARITGYIIKYEKPGSPPREVVPRPRPGVTEATITGLEPGTEYTIYVIALKNNQKSEPLIGRKKTDELPQLVTLPHPNLHGPEILDVPSTVQKTPFVTHPGYDTGNGIQLPGTSGQQPSVGQQMIFEEHGFRRTTPPTTATPIRHRPRPYPPNVGQEALSQTTISWAPFQDTSEYIISCHPVGTDEEPLQFRVPGTSTSATLTGLTRGATYNIIVEALKDQQRHKVREEVVTVGNSVNEGLNQPTDDSCFDPYTVSHYAVGDEWERMSESGFKLLCQCLGFGSGHFRCDSSRWCHDNGVNYKIGEKWDRQGENGQMMSCTCLGNGKGEFKCDPHEATCYDDGKTYHVGEQWQKEYLGAICSCTCFGGQRGWRCDNCRRPGGEPSPEGTTGQSYNQYSQRYHQRTNTNVNCPIECFMPLDVQADREDSRE

SEQ ID NO: 7 - protein, 109 aa, Homo sapiens
SLGSLTIAEPAMIAECKTRTEVFEISRRLIDRTNANFLVWPPCVEVQRCSGCCNNRNVQCRPTQVQLRPVQVRKIEIVRKKPIFKKATVTLEDHLACKCETVAAARPVT

SEQ ID NO: 8 - protein, 2179 aa, Homo sapiens
GVLKKVIRHKRQSGVNATLPEENQPVVFNHVYNIKLPVGSQCSVDLESASGEKDLAPPSEPSESFQEHTVDGENQIVFTHRINIPRRACGCAAAPDVKELLSRLEELENLVSSLREQCTAGAGCCLQPATGRLDTRPFCSGRGNFSTEGCGCVCEPGWKGPNCSEPECPGNCHLRGRCIDGQCICDDGFTGEDCSQLACPSDCNDQGKCVNGVCICFEGYAGADCSREICPVPCSEEHGTCVDGLCVCHDGFAGDDCNKPLCLNNCYNRGRCVENECVCDEGFTGEDCSELICPNDCFDRGRCINGTCYCEEGFTGEDCGKPTCPHACHTQGRCEEGQCVCDEGFAGVDCSEKRCPADCHNRGRCVDGRCECDDGFTGADCGELKCPNGCSGHGRCVNGQCVCDEGYTGEDCSQLRCPNDCHSRGRCVEGKCVCEQGFKGYDCSDMSCPNDCHQHGRCVNGMCVCDDGYTGEDCRDRQCPRDCSNRGLCVDGQCVCEDGFTGPDCAELSCPNDCHGQGRCVNGQCVCHEGFMGKDCKEQRCPSDCHGQGRCVDGQCICHEGFTGLDCGQHSCPSDCNNLGQCVSGRCICNEGYSGEDCSEVSPPKDLVVTEVTEETVNLAWDNEMRVTEYLVVYTPTHEGGLEMQFRVPGDQTSTIIQELEPGVEYFIRVFAILENKKSIPVSARVATYLPAPEGLKFKSIKETSVEVEWDPLDIAFETWEIIFRNMNKEDEGEITKSLRRPETSYRQTGLAPGQEYEISLHIVKNNTRGPGLKRVTTTRLDAPSQIEVKDVTDTTALITWFKPLAEIDGIELTYGIKDVPGDRTTIDLTEDENQYSIGNLKPDTEYEVSLISRRGDMSSNPAKETFTTGLDAPRNLRRVSQTDNSITLEWRNGKAAIDSYRIKYAPISGGDHAEVDVPKSQQATTKTTLTGLRPGTEYGIGVSAVKEDKESNPATINAATELDTPKDLQVSETAETSLTLLWKTPLAKFDRYRLNYSLPTGQWVGVQLPRNTTSYVLRGLEPGQEYNVLLTAEKGRHKSKPARVKASTEQAPELENLTVTEVGWDGLRLNWTAADQAYEHFIIQVQEANKVEAARNLTVPGSLRAVDIPGLKAATPYTVSIYGVIQGYRTPVLSAEASTGETPNLGEVVVAEVGWDALKLNWTAPEGAYEYFFIQVQEADTVEAAQNLTVPGGLRSTDLPGLKAATHYTITIRGVTQDFSTTPLSVEVLTEEVPDMGNLTVTEVSWDALRLNWTTPDGTYDQFTIQVQEADQVEEAHNLTVPGSLRSMEIPGLRAGTPYTVTLHGEVRGHSTRPLAVEVVTEDLPQLGDLAVSEVGWDGLRLNWTAADNAYEHFVIQVQEVNKVEAAQNLTLPGSLRAVDIPGLEAATPYRVSIYGVIRGYRTPVLSAEASTAKEPEIGNLNVSDITPESFNLSWMATDGIFETFTIEIIDSNRLLETVEYNISGAERTAHISGLPPSTDFIVYLSGLAPSIRTKTISATATTEALPLLENLTISDINPYGFTVSWMASENAFDSFLVTVVDSGKLLDPQEFTLSGTQRKLELRGLITGIGYEVMVSGFTQGHQTKPLRAEIVTEAEPEVDNLLVSDATPDGFRLSWTADEGVFDNFVLKIRDTKKQSEPLEITLLAPERTRDITGLREATEYEIELYGISKGRRSQTVSAIATTAMGSPKEVIFSDITENSATVSWRAPTAQVESFRITYVPITGGTPSMVTVDGTKTQTRLVKLIPGVEYLVSIIAMKGFEESEPVSGSFTTALDGPSGLVTANITDSEALARWQPAIATVDSYVISYTGEKVPEITRTVSGNTVEYALTDLEPATEYTLRIFAEKGPQKSSTITAKFTTDLDSPRDLTATEVQSETALLTWRPPRASVTGYLLVYESVDGTVKEVIVGPDTTSYSLADLSPSTHYTAKIQALNGPLRSNMIQTIFTTIGLLYPFPKDCSQAMLNGDTTSGLYTIYLNGDKAEALEVFCDMTSDGGGWIVFLRRKNGRENFYQNWKAYAAGFGDRREEFWLGLDNLNKITAQGQYELRVDLRDHGETAFAVYDKFSVGDAKTRYKLKVEGYSGTAGDSMAYHNGRSFSTFDKDTDSAITNCALSYKGAFWYRNCHRVNLMGRYGDNNHSQGVNWFHWKGHEHSIQFAEMKLRPSNFRNLEGRRKRA